European Patent Application EP 4 726 034 A1, published April 15, 2026. Title: CRISPR ribonucleoprotein complex with a type II-B Cas9 and the use thereof. Applicant: Consejo Superior de Investigaciones Cientificas (CSIC). Application EP. The sequence listing filed with the application follows.

SEQUENCE LISTING (60 sequences)

SEQ ID NO: 1 - protein, 1415 aa, unidentified
MTDSKIISPIAIDLGGLYTGLYMAQYPYGESLAQHHGKLTTLVMPEEGGKMTWSQAARTATRHRIRSNKRRKLAKRLLKVIFTQGLSYKLNDAELEALNGLLNRRGYNRVETDIDRQPLETVPPSWIANEFPEFFDSSSPISEQLEELLEDIPKLRDLAADEKFNLNNREAKKQLFTDAEDEQADILKAYGILRESVTELLNSIDFGHQHRRKYLEAVGKEILKDSRLAELRAKLGASALKNLIGNISNLQLRALRWYFNDTAMKSADYYDGERFKSVYVRWLQNWHVDEETRVNRNNALKVIHPSEDILTALMTIDAELTIPPYENQNNRRPPKDQTLWLNPQSLNEQYGSQWRVWVNNLRKRNPELAEGIAPVLEFTDRRSRLKTNKQRLTDTSLYADSYFLQRLLDRSRIHDTYALRAISKNFKSEKLEKFRWNLKQDLGDQHTEKFLDFTQKYYQEVERAKSGIWEQESASLLEKADINPPSKRKILNRLVGNILGVEMSAEELTTFLSDVWTKKVHGPSTVKSICKAAEDLRKQNGNLFNMYIQSVRYRASVEAGAEKKFKGLDKEIWQLLVKVEKAADVISGSISATETQKQRFSNTFSLAQLYTLIETDRNGFSKVSAAAHMELAWRMTMIPVDDKEAARCSRLPADSSRPFDGVLRRLLERQAYEIATLKSGQIKESGVRDSEISIPVVVEENRFTFSIGLADVKKDGSKRKKLLSLGEKQLEKWQEKNERIRQGGSGLCPYKGTILDKDAELDHIIPRSYSRDASGTIFNSEANLIYASRRGNQEKKDQRYGISDLAPNYLKAVYGTSDSAEITRIIEASVASIKKDFLFSELEGDQQRDVRHALFLERDSKAFEKVFRRLATQQSARVNGTQAWLARKLISVLKSQLKSWLSETGNTIVFNLCKADAQQTSFVRTGLAVTKPETTKGERQGVGSHAIDAYCAFSVAAAEGMHETLAQGAGLMEDTEWLATALPVDVDVNWVKRLPLYRKSELSTRPIFKEGIYAESFLTTWISEKGIESGFSLGSNSVQWQGKDTRGLLELLAPFATKNLNVDTALASPRPVQLDISKEKAFKHFEMVAKAPHSEVDLHQADILDALRYCTAKKDISSRLIDVQKKTLKKPEEVLKAKDIYVKVDVDVKGLGKLKGKVTHPAIEQWKRLFLIPDIETRIGEKAVGINWQQIGEKYFGEGSSRPHSKTRRVYSLPIVDSPDGGYRIKRIAPDGSTIWQLTSIKDTGSSGFTVNDKGVNWKQPVAIPALRDSSVVGVGERYQPVPEQQVYFDDWKCVDITDERVLSVSVAPGTKDRRYVSVSQTLSDFKAWLTESGIKLHSPFEIPSRVKVDAAKFQSAHGIDVLGKPKSNLFISKVGDVVNYWYIRESSPVVINQYYDKALLAEREAVNETEPCDI

SEQ ID NO: 2 - DNA, 4242 bp, unidentified
  source 1..4242: mol_type = genomic DNA
actgactctaaaatcatctctccaatcgcgattgacctcggtggtctttataccggtctgtatatggcgcaatatccgtatggagagagcctcgctcagcatcatggcaagctgacaacgctggttatgccagaagagggcggcaaaatgacctggtcgcaagcggcgcggactgctacccggcaccgcatacgttcaaacaaacgtagaaagctggcgaaacgtttactgaaagtgatctttactcaagggctgtcttacaagctgaatgatgcagaacttgaggccttgaatggcttgctgaatcgtagggggtacaacagagtagaaacggatattgatcgccaacctcttgagactgttcctccttcctggattgccaatgagttcccagaatttttcgatagtagcagtcctatatctgagcaattagaagaactactggaagacattcccaaacttcgtgatttggcggctgatgagaagtttaatcttaataatcgcgaagcaaagaagcagttatttacagacgcagaagacgaacaagcagatattctgaaagcctacggtattcttcgggaatcagtaacagagttgcttaacagtatcgacttcgggcaccagcatcgtcgaaaataccttgaagccgtaggtaaagagattttgaaggattcccgattagcagagctgcgggctaagctcggggcttccgccctcaagaatcttattggcaacatcagcaacctgcagttgcgagcgctaagatggtactttaacgataccgcgatgaagagtgccgattactatgatggcgaacgcttcaagtcggtatatgttcgttggctgcagaactggcatgtggacgaagaaacgcgagttaatcgcaacaatgcattaaaagtgattcatccttcagaagatattctcacggcgttgatgacgattgatgcagaactgacgattccaccctatgaaaatcagaataaccgtcgacctccaaaagatcagaccttatggcttaacccccagtcactgaatgagcaatatggctcacagtggcgtgtatgggttaataatctccgtaaacgtaatccggagctggcagagggaatcgcgcctgttcttgagttcactgaccgccgttcacgtttgaaaaccaataagcagcgcctgactgatacgtctttatatgcagacagctattttcttcagcgtcttcttgatcgcagcaggatccatgatacctacgcactccgtgcgatatcaaagaacttcaagtcagaaaaacttgaaaaattccgctggaacctgaagcaggatctgggagatcaacatacagaaaagtttctggacttcactcagaagtattaccaggaagtggaacgcgcaaaaagtggcatctgggagcaggaatcggcatcactgcttgaaaaagcggatattaaccctccctcaaagcgaaagattctgaatcgattagtagggaatattcttggcgttgaaatgagcgctgaagaactgaccacctttctgtcagacgtatggacgaagaaagttcatggcccatcaacggtaaagagtatctgcaaagctgccgaagacctgagaaaacagaatggcaacctcttcaatatgtatatccagtctgtacggtatcgagcgtcggtcgaagcaggtgcagagaagaaatttaaaggtctggataaagaaatttggcagcttctggttaaagtagagaaagcagcagatgtgatttctggttcaatttctgcgaccgaaacgcagaaacaaagattcagtaataccttttcacttgctcagttgtacaccctgatagagacagaccggaacggattctcaaaggtcagtgctgctgcacacatggagcttgcatggcgtatgacaatgataccggtggacgataaggaagccgcacgttgttcgcgcttgccagcagacagttctcggccattcgacggagtgttaagacgcttgctcgaacgtcaggcttatgaaatagcgacgctgaaatcggggcagataaaagagtccggtgtcagagactctgaaataagcattccagtggtggtagaagaaaaccgctttactttcagtattggccttgcagatgtaaaaaaagatggatcgaagcgaaaaaagctgctatcgctgggtgagaagcaactggaaaaatggcaagaaaagaatgaacgcatcagacagggcgggagtggcctgtgcccttataagggaacaattctggataaagatgctgagctagatcacataattccacgctcgtacagtcgtgatgcatcagggacaatcttcaatagcgaagccaatcttatttacgccagccgccgtggcaatcaggaaaagaaagaccaacgttacggcatttctgacttggcacccaattacctcaaggccgtctatgggacgtcagattcggcagagataacccggattatcgaagcgtctgtggcgtctattaagaaggacttcctcttctcagagctagaaggtgatcagcaaagggatgtccgccatgccttattcctggaacgtgattcaaaggcatttgagaaggtattcagacgcctggcaactcaacagagcgcgcgagtgaatggcacacaggcatggctggccagaaaactgatcagcgtattgaaaagccagttgaaatcctggctgtctgaaacgggtaatacgatcgtctttaacctgtgtaaagcagatgctcagcaaacatcgttcgttcgcaccgggcttgcagtgacaaagcctgagacaaccaaaggagagcgccagggtgtaggatctcacgccatcgatgcctattgtgcattctcagttgcagccgctgaaggcatgcacgaaacgctcgctcaaggcgcgggactcatggaggataccgagtggcttgcaacggcgttacctgttgacgttgatgtgaattgggttaaacgcctacctctatatcgcaagtcagaactaagtactcggccaatatttaaagaaggaatttatgcagagtcatttctgacgacctggatttcagagaaaggaattgaatccggcttctcattgggaagcaattcggtgcaatggcaaggtaaggatactcgtgggctacttgaattactggcaccattcgccactaaaaatttaaatgtcgataccgccctggcaagccctcgccctgtacagctagatattagtaaagaaaaagcgttcaagcacttcgaaatggtggccaaagcgccgcattcagaggtcgatctgcatcaggcggatattcttgatgctctcaggtattgcaccgcgaaaaaggatatcagttcgcgtctgattgatgtacagaagaaaacactgaaaaaaccagaggaagtgctaaaggctaaagatatttacgtgaaggttgatgttgacgttaaaggcctgggtaagttaaagggcaaggtcactcatccggcgattgagcaatggaaaagactattccttatcccggacatagagacacgcattggggaaaaagcggtaggcattaactggcaacaaattggtgaaaaatactttggtgaaggatcgtcccgcccacacagtaaaacgcgaagggtatattcgttacctatcgtcgatagccctgacggcggctatcgaattaaaagaatagcgcctgatggttcaacgatctggcaactgacgagtatcaaagatacgggatctagcgggtttacggtaaatgacaagggtgtaaattggaagcaaccagtggctatccctgcgctgcgtgattcttcggtcgttggggttggtgaacgttaccagcctgttcctgagcagcaagtatacttcgatgattggaaatgcgtagacataacggatgagcgtgtgttgtcagtctcagtggctcctggtactaaagatcggcgctatgtctcagtcagtcagactctatctgattttaaggcatggttaaccgagagtggtataaaactacattcgcctttcgaaattccctcaagagtcaaagtggatgctgctaaattccagtcggcacatggcattgacgtactaggaaaaccgaaatcgaatttgtttatttcgaaggtcggggatgtcgttaactattggtacatcagagaaagtagtcctgttgtgattaatcagtattacgacaaggcactcctggcagagcgcgaagcagttaacgagaccgagccatgcgacatc

SEQ ID NO: 3 - RNA, 37 nt, unidentified
  source 1..37: mol_type = other RNA
gtttcagttgcaggtttattgggataggctttgcaac

SEQ ID NO: 4 - RNA, 104 nt, unidentified
  source 1..104: mol_type = other RNA; note = ANTISENSE_RNA
tttttctttttggggcctacggcttcgtccacggcctcagtcagtactaaaatctactaaagtcgagcgggcacccgctgaagttagtccggataaccctatcc

SEQ ID NO: 5 - RNA, 136 nt, synthetic construct
  source 1..136: mol_type = other RNA
gtttcagttgcaggtttattgggatagggaaacctatcccaataggcctgattgaagtcgcccacgggcgagctgaaatcatctaaaatcatgactgactccggcacctgcttcggcatccggggtttttcttttt

SEQ ID NO: 6 - DNA, 20 bp, Homo sapiens
  source 1..20: mol_type = genomic DNA
tccaaggtgaaagcggaagt

SEQ ID NO: 7 - DNA, 20 bp, Homo sapiens
  source 1..20: mol_type = genomic DNA
gaagagggtgcattttcagg

SEQ ID NO: 8 - DNA, 20 bp, Homo sapiens
  source 1..20: mol_type = genomic DNA
gcttcgtggcaatgcgccac

SEQ ID NO: 9 - DNA, 20 bp, Homo sapiens
  source 1..20: mol_type = genomic DNA
gaccccctccaccccgcctc

SEQ ID NO: 10 - DNA, 20 bp, Homo sapiens
  source 1..20: mol_type = genomic DNA
gggaaaggtaatcgaactgt

SEQ ID NO: 11 - DNA, 20 bp, synthetic construct
  source 1..20: mol_type = other DNA
ggaatcccttctgcagcacc

SEQ ID NO: 12 - DNA, 21 bp, synthetic construct
  source 1..21: mol_type = other DNA
ccgaaaaagaagcgaaaggtc

SEQ ID NO: 13 - DNA, 4311 bp, synthetic construct
  source 1..4311: mol_type = other DNA
ccgaaaaagaagcgaaaggtcaccgactcaaaaatcatcagccctattgccatcgatctcggcggcctgtacaccggtctctacatggcccagtacccttacggcgaaagcctggcccagcaccacggcaagctcacaacactggtgatgcctgaagaaggcggcaagatgacctggagccaggccgctagaacagccacccggcacaggatcagaagcaacaagcggagaaagctggccaagagactgctgaaggtgatcttcacccagggcctgagctacaagctgaatgacgccgagctggaggccctgaatggcctgctgaacaggaggggctacaacagagttgagaccgacatcgatcggcagcctctggagaccgtgcccccttcttggatcgccaatgagttccccgaattcttcgacagctctagccctatcagcgagcagctggaggaactgctcgaggacatccccaagttaagggacctggctgctgatgaaaagttcaatctgaacaaccgggaagccaagaaacagctgtttacagacgccgaggatgagcaggcagatatcctgaaggcttatggcatcctgcgggaatctgtgaccgagctgttaaacagcatcgactttggacaccagcacagacggaaatacctggaggccgtgggcaaggagatcctgaaagatagcagactggccgaacttagagccaaactgggcgccagcgccctgaagaacctgataggaaacatcagcaacctgcagctacgggccctgaggtggtattttaatgataccgccatgaagagtgctgactactacgacggcgaaagattcaagagcgtgtacgtgagatggctgcaaaactggcacgtagacgaggaaacgcgggtgaacaggaacaacgccctgaaggtgatccacccaagcgaggacatcctgacagctctgatgaccatcgacgccgagctgactatccctccttacgagaaccagaacaaccggagaccacctaaggaccagaccctgtggctgaatccccagagcctgaatgaacaatacggctctcagtggcgggtgtgggtcaacaacctgagaaaacggaaccccgagctggccgaaggcatcgcccctgtgctggagttcacagacagaagaagcaggcttaagacaaacaagcagagactgacagacacctctctgtacgctgacagctacttcctgcagcggctcctcgaccggagccgcattcacgacacctacgccctcagagcaatctccaaaaacttcaagagtgaaaagctggagaaattccggtggaacctgaagcaggacctgggcgaccagcataccgagaagttcctggatttcacccaaaagtactatcaggaggtggaaagagctaagtctggcatctgggagcaggaatctgcgtctctcctggaaaaggcggatatcaaccctccaagcaagcggaagatcctcaatcgcctggtcggaaatatcctgggcgtggaaatgagcgccgaagagctgaccaccttcctgtctgatgtgtggaccaaaaaggtgcacggccctagcaccgtgaagagcatctgcaaggccgccgaggacctgcgcaagcaaaacggcaacctgttcaacatgtacatccagagcgtgagataccgggccagtgtggaagctggcgctgagaagaaattcaaaggcctggacaaagagatctggcaactgctggtgaaagttgagaaggccgccgatgtgatcagcggaagcatcagcgccacagaaacccagaagcagagattcagcaataccttcagcctggcccagctgtacaccctgattgagacggacagaaacggcttcagcaaggtgtccgccgcggcccacatggaactggcctggagaatgacaatgatccccgtggatgacaaagaggccgcccggtgcagcaggttgcctgctgattctagcaggccctttgatggcgtgctgcgcagactgctggagcggcaagcctacgagatcgccacactgaagtccggccagatcaaggaaagcggcgtgagagacagcgagatcagcatccccgtggtcgtcgaggaaaaccggtttacctttagcatcggactggctgatgtgaaaaaagatggctccaaaagaaagaagctgctgtctctgggagaaaagcagctggagaagtggcaggagaagaacgagagaattagacagggaggcagcggactgtgtccttacaagggcaccatcctggacaaggatgccgagctggaccacatcatcccccggagctacagcagagacgccagcggcacaatcttcaactctgaggccaacctgatctacgccagccggagaggcaatcaggagaagaaggaccaacggtacggcatctccgatctggcccctaactacctgaaggccgtgtacggaaccagcgatagcgccgagatcaccagaattatcgaggcctccgtggcttctatcaagaaagacttcctgttcagcgagcttgaaggcgaccagcaacgggatgtgcgacatgccctgtttctggaaagagatagcaaggctttcgagaaagtgttcagacgtcttgctacacagcagagcgccagagtgaatggcacccaggcttggctcgccagaaagctgatctccgtgctgaagagccagctgaagtcctggctgtctgaaacaggcaacaccatcgtgttcaacctgtgcaaggccgatgctcaacagacatcattcgtccggaccggcctggctgtgaccaagcccgagacaaccaagggcgagagacagggcgtgggcagccacgccatcgacgcctactgcgccttctcggtcgccgccgccgagggcatgcacgagaccctggcccagggggccggcctgatggaagataccgagtggcttgctacagccctgcctgtggacgtggatgtgaactgggtgaagagactgcctctgtacagaaaatctgaattgagcacccggcccatcttcaaggaaggcatctatgctgaatcttttctgacaacctggatctctgagaagggcatcgagagcggattcagcctcggcagcaattctgtgcagtggcagggcaaggatacccggggtcttctggaactgctggccccttttgccaccaagaacctgaacgtggacaccgccctggcctcccctagacccgtgcagctggacatcagcaaggagaaggcctttaagcacttcgagatggtggccaaggccccgcactctgaagtggacctgcaccaggccgacatcctggacgccctgagatattgtacagccaagaaggacatctccagcagactgatcgacgtccagaagaagaccctaaagaaacctgaagaggtgctgaaggccaaggacatctacgtgaaagtggacgtggacgtaaagggcctggggaaactgaaaggcaaggtgacccaccccgctatcgagcagtggaagagactgttcctgatcccagatattgagacaagaatcggcgagaaggccgtgggcatcaactggcagcagatcggcgagaagtacttcggcgaaggctcctctcggccccatagcaagaccagaagggtttacagcctgccaatcgtggactctcctgatggaggataccggatcaaaagaatcgcccctgacggctcaaccatctggcagctgacaagcatcaaggacacaggatccagcggtttcaccgtgaacgacaagggcgtgaactggaagcagcctgttgccatccctgccctgagagatagcagcgtggtgggcgtgggcgagagataccagccagtgcctgagcagcaggtgtacttcgacgactggaagtgcgtggacattacagacgagagagtgctgtccgtgagcgtggcccctggtacaaaggacagacggtacgtgagcgttagccagaccctgagcgatttcaaggcatggctgaccgagagcgggatcaagctgcacagccccttcgagatcccaagccgggtcaaagtggacgccgctaagtttcagagcgcccatggcatcgacgtgctgggcaagcctaagagcaacctgttcatctctaaggtcggagatgtggtgaactactggtacatcagagaatcctcccctgtggtcataaaccagtactacgacaaggctctgctggccgaaagagaggctgtgaacgagaccgagccctgcgacatcaaaaggccggcggccacgaaaaaggccggccaggcaaaaaagaaaaag

SEQ ID NO: 14 - DNA, 21 bp, synthetic construct
  source 1..21: mol_type = other DNA
ccgaagaagaaacgaaaagtt

SEQ ID NO: 15 - DNA, 4326 bp, synthetic construct
  source 1..4326: mol_type = other DNA
atgaagattgaggagacggatagtaagataattagtcctatagccatagatcttggtggactctacacaggcctttacatggcacagtacccttacggtgaaagtctggcacaacaccacggtaaattgacgactttggtcatgccggaagaaggcggaaagatgacttggagccaggcagcccgcacggccacacgccatagaattcgctccaataagcgccgcaaactcgctaagcgcctcttgaaggttattttcacacagggcttaagctataaactcaacgacgccgagttagaagctctgaacgggctgcttaacagaagaggttataatcgggttgagacagacatcgaccgacagcccctggaaacggtgcccccaagctggatcgcaaacgaatttcctgagttctttgactcctcttcaccgatcagtgaacagttagaggagttattagaggatatcccgaagctccgcgacctggccgcggacgagaaattcaacctgaacaaccgggaagcgaagaagcaacttttcaccgatgctgaggatgagcaggcggacatactcaaggcatatggcatcctgcgtgagtccgtgaccgaactcctgaatagcattgattttggtcatcaacaccggcgtaagtatttagaggcggtgggcaaggaaatcctgaaagactctcgtctggccgaattacgcgcaaaactgggcgccagcgctcttaagaacctgatcgggaatataagtaatcttcaactccgtgcattgcggtggtatttcaatgacacggccatgaaatctgcagactattacgacggggagagatttaaatctgtctacgtgcgctggctccaaaattggcacgtagatgaggagactcgtgtcaacagaaataacgcgcttaaggtcatccacccaagtgaggacatactgacagctctgatgactatcgacgcggagctcactatcccgccttacgagaaccaaaacaatcgccgcccgccgaaggaccaaactctgtggttgaatccgcaatctttgaacgaacagtacgggtcgcaatggcgcgtgtgggtcaacaacctgcgaaagagaaaccctgaattagctgaaggcattgccccggtattggaatttacagatagacgctctcggctgaagacgaacaaacaacgtttaacggacacttcactttacgccgattcctacttcctgcaacgcttgctggacagaagtcgtattcacgacacgtatgcgcttcgcgctatttcgaagaattttaaaagcgagaagttagagaagtttcgatggaatctcaaacaagacctcggtgaccagcacacggagaaattcttagattttacgcagaaatactatcaagaggtcgagcgtgctaagtctggaatttgggaacaagagagtgcctctttgctcgaaaaggccgacataaatccgccgtccaaacgtaaaatactcaaccgcttggttggaaacatcctgggagtagagatgtccgccgaggagcttactacattcttgtctgatgtttggaccaagaaggtacacggtccatccactgttaaatctatatgtaaggcagctgaggatttgcgtaagcaaaacggtaatctgtttaacatgtacattcaaagtgtcagataccgggcctcagtagaggctggggctgagaagaagttcaagggcttagacaaggagatctggcaactgttagtgaaggttgaaaaggctgccgacgttatcagcggatctatcagcgcaacagagacccaaaagcagcgtttctcaaacacattcagcttagcccaactttatacgttaattgaaaccgatcgaaatggcttttccaaagtgtcggcagcagcgcatatggaattagcttggagaatgactatgatcccagttgatgacaaagaggcggcgcgatgctcaagattacctgctgattcttcgagaccgtttgatggtgttcttcgccgtctgttggagcgacaagcatacgagattgcaacattgaagtctggccaaattaaggaaagcggcgtgcgcgattccgagatttctatcccggttgttgtggaagagaatcgtttcacctttagcatcgggttagccgacgttaagaaggacggtagtaaaagaaagaaattactgagtcttggagaaaagcagctcgaaaagtggcaggagaagaacgagagaattcgtcaaggtggtagcggactctgtccctacaaagggactatcctcgacaaggacgcggaactggaccatattataccgcgttcttattcgcgagacgccagtggtactatatttaacagtgaggcgaacctgatctatgcaagtcgtcgcggaaaccaagagaagaaggatcagagatatggaatctccgatctggctccaaactatctgaaagcggtgtacggcacaagcgacagtgctgaaattactcgtatcattgaggcatccgtagcaagcatcaagaaagattttctgtttagtgaattagagggcgaccaacagcgtgacgtacgtcacgcgctctttcttgagcgggactctaaagcgttcgagaaagtatttcgtcggcttgcgacccagcaatcagcacgcgttaacgggacgcaagcttggcttgcgcgaaagcttatttcggtgcttaagtctcaactcaagtcatggctttccgagaccggcaacacaatagttttcaatttatgcaaggccgacgcacaacagacctcttttgtccgtacgggattggctgttaccaaaccggaaaccactaagggcgaacggcaaggcgtgggctcacatgctattgacgcatactgcgccttttctgtggccgcggccgagggtatgcatgagacactggcacagggtgccgggcttatggaagacacagaatggttagctacagccctgccagtggatgtggacgtcaactgggtcaagcgtctgccgctgtaccgaaaatctgagctgtcaacccgtcctattttcaaagagggcatatacgccgaaagtttcttaaccacatggatatcggaaaagggtatagagagcggcttttctctgggctcaaacagtgtccagtggcagggaaaagacacacgaggtctgttagagttgttggctccgtttgctacgaagaacctgaacgtggacactgcactcgcgtcaccgcgtccggtgcaattggacatatcgaaggagaaggcatttaaacattttgagatggtagctaaggccccacacagtgaagtagacttacaccaagcagacatcctggacgcactgcgctactgtacggctaagaaagacattagcagccgattaatcgacgtgcaaaagaagacccttaagaagcctgaagaggttttaaaagcgaaggacatctatgttaaagtggacgtggatgtgaaggggcttggcaaactgaaaggaaaagttacccacccagccatagaacagtggaagcgtctgtttcttattccagatattgaaacccgtatcggtgagaaggcagtcggtataaattggcagcagataggcgagaagtatttcggcgagggtagcagtcgtccccattctaagactcgtcgcgtctactcactgccgattgttgactctccagatggtggttaccgcataaagcgtatcgccccagacggcagtactatttggcagttaacaagcattaaggacacagggtcctctggattcactgtcaacgataaaggggttaactggaaacagcctgtagcaataccggccttacgggactccagcgtggtaggcgtcggcgagcgctatcaaccggtgccggaacaacaggtgtattttgacgactggaagtgtgttgatatcacagacgaaagagttctgagtgtatcggtagcgccgggcaccaaggaccgacgttacgtttctgtgtcacaaacgctttcggacttcaaagcgtggctcacggaatccggcatcaagctgcacagcccgtttgagataccgtcccgcgttaaggtcgacgccgccaagtttcaaagcgcccacggaatcgatgtccttggtaagcccaagagtaacttattcatctccaaagtgggcgacgttgtcaattactggtatattcgggagtcttcgccggtagttataaaccaatactatgataaagccttgcttgcggaacgcgaggccgtgaatgaaacggaaccttgtgatatatctcgtgcggacccgaagaagaaacgaaaagttgctgctgctctcgagcaccaccaccaccaccactga

SEQ ID NO: 16 - DNA, 179 bp, synthetic construct
  source 1..179: mol_type = other DNA
aagctaatacgactcactatagggctaccataggcaccacgaggtttcagttgcaggtttattgggatagggaaacctatcccaataggcctgattgaagtcgcccacgggcgagctgaaatcatctaaaatcatgactgactccggcacctgcttcggcatccggggtttttcttttt

SEQ ID NO: 17 - DNA, 125 bp, synthetic construct
  source 1..125: mol_type = other DNA
aaagcaagcaagctaatacgactcactatagggctaccataggcaccacgaggtttcagttgcgccgaaaggcgctctgtaatcatttaaaagtattttgaacggacctctgtttgacacgtctg

SEQ ID NO: 18 - DNA, 44 bp, synthetic construct
  source 1..44: mol_type = other DNA
ggcaagatatgtccgatattgatttgcgccgaattttctgaaat

SEQ ID NO: 19 - DNA, 44 bp, synthetic construct
  source 1..44: mol_type = other DNA
ggcaagatatgtccgatatcgatttgcgccgaattttctgaaat

SEQ ID NO: 20 - DNA, 179 bp, synthetic construct
  source 1..179: mol_type = other DNA
aagctaatacgactcactataggaattcggcgcaaatcaatatgtttcagttgcaggtttattgggatagggaaacctatcccaataggcctgattgaagtcgcccacgggcgagctgaaatcatctaaaatcatgactgactccggcacctgcttcggcatccggggtttttcttttt

SEQ ID NO: 21 - DNA, 123 bp, synthetic construct
  source 1..123: mol_type = other DNA
aagctaatacgactcactataggaattcggcgcaaatcgatatgttttagagctagaaatagcaagttaaaataaggctagtccgttatcaacttgaaaaagtggcaccgagtcggtgctttt

SEQ ID NO: 22 - DNA, 135 bp, synthetic construct
  source 1..135: mol_type = other DNA
aagctaatacgactcactataggctaccataggcaccacgaggtttaagagctatgctggaaacagcatagcaagtttaaataaggctagtccgttatcaacttgaaaaagtggcaccgagtcggtgcttttttt

SEQ ID NO: 23 - DNA, 135 bp, synthetic construct
  source 1..135: mol_type = other DNA
aagctaatacgactcactataggctaccataggcaccacgacgtttaagagctatgctggaaacagcatagcaagtttaaataaggctagtccgttatcaacttgaaaaagtggcaccgagtcggtgcttttttt

SEQ ID NO: 24 - DNA, 135 bp, synthetic construct
  source 1..135: mol_type = other DNA
aagctaatacgactcactataggctaccataggcaccacaaggtttaagagctatgctggaaacagcatagcaagtttaaataaggctagtccgttatcaacttgaaaaagtggcaccgagtcggtgcttttttt

SEQ ID NO: 25 - DNA, 135 bp, synthetic construct
  source 1..135: mol_type = other DNA
aagctaatacgactcactataggctaccataggcacctcgaggtttaagagctatgctggaaacagcatagcaagtttaaataaggctagtccgttatcaacttgaaaaagtggcaccgagtcggtgcttttttt

SEQ ID NO: 26 - DNA, 179 bp, synthetic construct; identical to SEQ ID NO: 16
  source 1..179: mol_type = other DNA

SEQ ID NO: 27 - DNA, 179 bp, synthetic construct
  source 1..179: mol_type = other DNA
aagctaatacgactcactatagggctaccataggcaccacgacgtttcagttgcaggtttattgggatagggaaacctatcccaataggcctgattgaagtcgcccacgggcgagctgaaatcatctaaaatcatgactgactccggcacctgcttcggcatccggggtttttcttttt

SEQ ID NO: 28 - DNA, 179 bp, synthetic construct
  source 1..179: mol_type = other DNA
aagctaatacgactcactatagggctaccataggcaccacaaggtttcagttgcaggtttattgggatagggaaacctatcccaataggcctgattgaagtcgcccacgggcgagctgaaatcatctaaaatcatgactgactccggcacctgcttcggcatccggggtttttcttttt

SEQ ID NO: 29 - DNA, 179 bp, synthetic construct
  source 1..179: mol_type = other DNA
aagctaatacgactcactatagggctaccataggcacctcgaggtttcagttgcaggtttattgggatagggaaacctatcccaataggcctgattgaagtcgcccacgggcgagctgaaatcatctaaaatcatgactgactccggcacctgcttcggcatccggggtttttcttttt

SEQ ID NO: 30 - DNA, 173 bp, synthetic construct
  source 1..173: mol_type = other DNA
taatacgactcactataggggaaggttgattatgcacgtttcagttgcaggtttattccctatccctttggatagggttatccggactaacttcagcgggtgcccgctcgactttagtagattttagtactgactgaggccgtggacgaagccgtaggccccaaaaagaaaaa

SEQ ID NO: 31 - DNA, 173 bp, synthetic construct
  source 1..173: mol_type = other DNA
taatacgactcactataggagcctccgaggcgctctagtttcagttgcaggtttattccctatccctttggatagggttatccggactaacttcagcgggtgcccgctcgactttagtagattttagtactgactgaggccgtggacgaagccgtaggccccaaaaagaaaaa

SEQ ID NO: 32 - DNA, 173 bp, synthetic construct
  source 1..173: mol_type = other DNA
taatacgactcactatagggtccgtcaatgaagtctggtttcagttgcaggtttattccctatccctttggatagggttatccggactaacttcagcgggtgcccgctcgactttagtagattttagtactgactgaggccgtggacgaagccgtaggccccaaaaagaaaaa

SEQ ID NO: 33 - DNA, 13180 bp, synthetic construct
  source 1..13180: mol_type = other DNA
tgagacgaagctttgacaggatatattggcgggtaaacctaagagaaaagagcgtttattagaataatcggatatttaaaagggcgtgaaaaggtttatccgttcgtccatttgtatgtgcatgccaaccacagggttcccctcgggatcaaagtactttgatccaacccctccgctgctatagtgcagtcggcttctgacgttcagtgcagccgtcatctgaaaacgacatgtcgcacaagtcctaagttacgcgacaggctgccgccctgcccttttcctggcgttttcttgtcgcgtgttttagtcgcataaagtagaatacttgcgactagaaccggagacattacgccatgaacaagagcgccgccgctggcctgctgggctatgcccgcgtcagcaccgacgaccaggacttgaccaaccaacgggccgaactgcacgcggccggctgcaccaagctgttttccgagaagatcaccggcaccaggcgcgaccgcccggagctggccaggatgcttgaccacctacgccctggcgacgttgtgacagtgaccaggctagaccgcctggcccgcagcacccgcgacctactggacattgccgagcgcatccaggaggccggcgcgggcctgcgtagcctggcagagccgtgggccgacaccaccacgccggccggccgcatggtgttgaccgtgttcgccggcattgccgagttcgagcgttccctaatcatcgaccgcacccggagcgggcgcgaggccgccaaggcccgaggcgtgaagtttggcccccgccctaccctcaccccggcacagatcgcgcacgcccgcgagctgatcgaccaggaaggccgcaccgtgaaagaggcggctgcactgcttggcgtgcatcgctcgaccctgtaccgcgcacttgagcgcagcgaggaagtgacgcccaccgaggccaggcggcgcggtgccttccgtgaggacgcattgaccgaggccgacgccctggcggccgccgagaatgaacgccaagaggaacaagcatgaaaccgcaccaggacggccaggacgaaccgtttttcattaccgaagagatcgaggcggagatgatcgcggccgggtacgtgttcgagccgcccgcgcacctctcaaccgtgcggctgcatgaaatcctggccggtttgtctgatgccaagctggcggcctggccggccagcttggccgctgaagaaaccgagcgccgccgtctaaaaaggtgatgtgtatttgagtaaaacagcttgcgtcatgcggtcgctgcgtatatgatccgatgagtaaataaacaaatacgcaaggggaacgcatgaaggttatcgctgtacttaaccagaaaggcgggtcaggcaagacgaccatcggaacccatctagcccgcgccctgcaactcgccggggccgatgttctgttagtcgattccgatccccagggcagtgcccgcgattgggcggccgtgcgggaagatcaaccgctaaccgttgtcggcatcgaccgcccgacgattgaccgcgacgtgaaggccatcggccggcgcgacttcgtagtgatcgacggagcgccccaggcggcggacttggctgtgtccgcgatcaaggcagccgacttcgtgctgattccggtgcagccaagcccttacgacatatgggccaccgccgacctggtggagctggttaagcagcgcattgaggtcacggatggaaggctacaagcggcctttgtcgtgtcgcgggcgatcaaaggcacgcgcatcggcggtgaggttgccgaggcgctggccgggtacgagctgcccattcttgagtcccgtatcacgcagcgcgtgagctacccaggcactgccgccgccggcacaaccgttcttgaatcagaacccgagggcgacgctgcccgcgaggtccaggcgctggccgctgaaattaaatcaaaactcatttgagttaatgaggtaaagagaaaatgagcaaaagcacaaacacgctaagtgccggccgtccgagcgcacgcagcagcaaggctgcaacgttggccagcctggcagacacgccagccatgaagcgggtcaactttcagttgccggcggaggatcacaccaagctgaagatgtacgcggtacgccaaggcaagaccattaccgagctgctatctgaatagatcgcgcagctaccagagtaaatgagcaaatgaataaatgagtagatgaattttagcggctaaaggaggcggcatggaaaatcaagaacaaccaggcaccgacgccgtggaatgccccatgtgtggaggaacgggcggttggccaggcgtaagcggctgggttgtctgccggccctgcaatggcactggaacccccaagcccgaggaatcggcgtgacggtcgcaaaccatccggcccggtacaaatcggcgcggcgctgggtgatgacctggtggagaagttgaaggccgcgcaggccgcccagcggcaacgcatcgaggcagaagcacgccccggtgaatcgtggcaagcggccgctgatcgaatccgcaaagaatcccggcaaccgccggcagccggtgcgccgtcgattaggaagccgcccaagggcgacgagcaaccagattttttcgttccgatgctctatgacgtgggcacccgcgatagtcgcagcatcatggacgtggccgttttccgtctgtcgaagcgtgaccgacgagctggcgaggtgatccgctacgagcttccagacgggcacgtagaggtttccgcagggccggccggcatggccagtgtgtgggattacgacctggtactgatggcggtttcccatctaaccgaatccatgaaccgataccgggaagggaagggagacaagcccggccgcgtgttccgtccacacgttgcggacgtactcaagttctgccggcgagccgatggcggaaagcagaaagacgacctggtagaaacctgcattcggttaaacaccacgcacgttgccatgcagcgtacgaagaaggccaagaacggccgcctggtgacggtatccgagggtgaagccttgattagccgctacaagatcgtaaagagcgaaaccgggcggccggagtacatcgagatcgagctagctgattggatgtaccgcgagatcacagaaggcaagaacccggacgtgctgacggttcaccccgattactttttgatcgatcccggcatcggccgttttctctaccgcctggcacgccgcgccgcaggcaaggcagaagccagatggttgttcaagacgatctacgaacgcagtggcagcgccggagagttcaagaagttctgtttcaccgtgcgcaagctgatcgggtcaaatgacctgccggagtacgatttgaaggaggaggcggggcaggctggcccgatcctagtcatgcgctaccgcaacctgatcgagggcgaagcatccgccggttcctaatgtacggagcagatgctagggcaaattgccctagcaggggaaaaaggtcgaaaaggactctttcctgtggatagcacgtacattgggaacccaaagccgtacattgggaaccggaacccgtacattgggaacccaaagccgtacattgggaaccggtcacacatgtaagtgactgatataaaagagaaaaaaggcgatttttccgcctaaaactctttaaaacttattaaaactcttaaaacccgcctggcctgtgcataactgtctggccagcgcacagccgaagagctgcaaaaagcgcctacccttcggtcgctgcgctccctacgccccgccgcttcgcgtcggcctatcgcggccgctggccgctcaaaaatggctggcctacggccaggcaatctaccagggcgcggacaagccgcgccgtcgccactcgaccgccggcgcccacatcaaggcaccctgcctcgcgcgtttcggtgatgacggtgaaaacctctgacacatgcagctcccggtgacggtcacagcttgtctgtaagcggatgccgggagcagacaagcccgtcagggcgcgtcagcgggtgttggcgggtgtcggggcgcagccatgacccagtcacgtagcgatagcggagtgtatactggcttaactatgcggcatcagagcagattgtactgagagtgcaccatatgcggtgtgaaataccgcacagatgcgtaaggagaaaataccgcatcaggcgctcttccgcttcctcgctcactgactcgctgcgctcggtcgttcggctgcggcgagcggtatcagctcactcaaaggcggtaatacggttatccacagaatcaggggataacgcaggaaagaacatgtgagcaaaaggccagcaaaaggccaggaaccgtaaaaaggccgcgttgctggcgtttttccataggctccgcccccctgacgagcatcacaaaaatcgacgctcaagtcagaggtggcgaaacccgacaggactataaagataccaggcgtttccccctggaagctccctcgtgcgctctcctgttccgaccctgccgcttaccggatacctgtccgcctttctcccttcgggaagcgtggcgctttctcatagctcacgctgtaggtatctcagttcggtgtaggtcgttcgctccaagctgggctgtgtgcacgaaccccccgttcagcccgaccgctgcgccttatccggtaactatcgtcttgagtccaacccggtaagacacgacttatcgccactggcagcagccactggtaacaggattagcagagcgaggtatgtaggcggtgctacagagttcttgaagtggtggcctaactacggctacactagaaggacagtatttggtatctgcgctctgctgaagccagttaccttcggaaaaagagttggtagctcttgatccggcaaacaaaccaccgctggtagcggtggtttttttgtttgcaagcagcagattacgcgcagaaaaaaaggatctcaagaagatcctttgatcttttctacggggtctgacgctcagtggaacgaaaactcacgttaagggattttggtcatgcattctaggtgattagaaaaactcatcgagcatcaaatgaaactgcaatttattcatatcaggattatcaataccatatttttgaaaaagccgtttctgtaatgaaggagaaaactcaccgaggcagttccataggatggcaagatcctggtatcggtctgcgattccgactcgtccaacatcaatacaacctattaatttcccctcgtcaaaaataaggttatcaagtgagaaatcaccatgagtgacgactgaatccggtgagaatggcaaaagtttatgcatttctttccagacttgttcaacaggccagccattacgctcgtcatcaaaatcactcgcatcaaccaaaccgttattcattcgtgattgcgcctgagcgagtcgaaatacgcgatcgctgttaaaaggacaattacaaacaggaatcgaatgcaaccggcgcaggaacactgccagcgcatcaacaatattttcacctgaatcaggatattcttctaatacctggaatgctgttttccctgggatcgcagtggtgagtaaccatgcatcatcaggagtacggataaaatgcttgatggtcggaagaggcataaattccgtcagccagtttagtctgaccatctcatctgtaacatcattggcaacgctacctttgccatgtttcagaaacaactctggcgcatcgggcttcccatacaatcggtagattgtcgcacctgattgcccgacattatcgcgagcccatttatacccatataaatcagcatccatgttggaatttaatcgcggccttgagcaagacgtttcccgttgaatatggctcataacagaacttattatttccttcctcttttctacagtatttaaagataccccaagaagctaattataacaagacgaactccaattcactgttccttgcattctaaaaccttaaataccagaaaacagctttttcaaagttgttttcaaagttggcgtataacatagtatcgacggagccgattttgaaaccgcggtgatcacaggcagcaacgctctgtcatcgttacaatcaacatgctaccctccgcgagatcatccgtgtttcaaacccggcagcttagttgccgttcttccgaatagcatcggtaacatgagcaaagtctgccgccttacaacggctctcccgctgacgccgtcccggactgatgggctgcctgtatcgagtggtgattttgtgccgagctgccggtcggggagctgttggctggctggtggcaggatatattgtggtgtaaacataacaagcttcgtctcagtcaggagactagagccaagctgatctcctttgccccggagatcaccatggacgactttctctatctctacgatctaggaagaaagttcgacggagaaggtgacgataccatgttcaccaccgataatgagaagattagcctcttcaatttcagaaagaatgctgacccacagatggttagagaggcctacgcggcaggtctgatcaagacgatctacccgagtaataatctccaggagatcaaataccttcccaagaaggttaaagatgcagtcaaaagattcaggactaactgcatcaagaacacagagaaagatatatttctcaagatcagaagtactattccagtatggacgattcaaggcttgcttcataaaccaaggcaagtaatagagattggagtctctaagaaagtagttcctactgaatcaaaggccatggagtcaaaaattcagatcgaggatctaacagaactcgccgtgaagactggcgaacagttcatacagagtcttttacgactcaatgacaagaagaaaatcttcgtcaacatggtggagcacgacactctcgtctactccaagaatatcaaagatacagtctcagaagaccaaagggctattgagacttttcaacaaagggtaatatcgggaaacctcctcggattccattgcccagctatctgtcacttcatcaaaaggacagtagaaaaggaaggtggcacctacaaatgccatcattgcgataaaggaaaggctatcgttcaagatgcctctgccgacagtggtcccaaagatggacccccacccacgaggagcatcgtggaaaaagaagacgttccaaccacgtcttcaaagcaagtggattgatgtgatatctccactgacgtaagggatgacgcacaatcccactatccttcgcaatgagacttttcaacaaagggtaatatcgggaaacctcctcggattccattgcccagctatctgtcacttcatcaaaaggacagtagaaaaggaaggtggcacctacaaatgccatcattgcgataaaggaaaggctatcgttcaagatgcctctgccgacagtggtcccaaagatggacccccacccacgaggagcatcgtggaaaaagaagacgttccaaccacgtcttcaaagcaagtggattgatgtgatatctccactgacgtaagggatgacgcacaatcccactatccttcgcaagacccttcctctatataaggaagttcatttcatttggagaggactccggtatttttacaacaattaccacaacaaaacaaacaacaaacaacattacaatttactattctagtcgaaatgcctaagaaaaaacgtaaggttagtatcatatgaagaaatacctagtttcagttgatgaatgctattttctgacctcagttgttctcttttgagaattatttcttttctaatttgcctgatttttctattaattcattaggtgaccgatagcaagattatcagcccgatcgcaattgatcttggaggcctctacacgggcctttacatggctcaatacccatacggagaatcactcgctcagcatcatgggaagctgacaacattggtcatgcccgaagaaggcggaaaaatgacttggtcacaggcagccagaacggccacccgtcatcgaatccgaagcaataaaagacgaaagctcgcaaagcgactgcttaaagtcatcttcacacagggcctttcctataaattgaacgacgcagaattagaggtaaatcctggtccacacttttacgataaaaacacaagattttaaactatgaactgatcaataatcattcctaaaagaccacacttttgttttgtttctaaagtaatttttactgttataacaggtcctgaatgggctcctgaacaggcgagggtataaccgagttgaaaccgatattgatcgacaacccttggaaactgtcccccccagttggatagcaaacgaattccctgagttcttcgactcttctagccccatatctgaacagctcgaggaattgctggaggacattcccaaactcagagatcttgccgccgatgagaaatttaatttaaacaatagggaggccaaaaaacagttatttactgacgccgaagatgagcaggctgacatattaaaagcttacggcatattgcgagagtctgtgactgagcttttgaacagcattgacttcggacatcaacaccgaagaaagtatcttgaagccgtgggcaaggaaatattgaaagatagccgtctggccgaactcagagcaaaacttggggccagtgcacttaagaatttaatcgggaatatcagcaacttgcaactgcgtgctcttcgttggtattttaacgatacagctatgaaatccgccgactattatgacggagagcgtttcaaatctgtctacgtcaggtaaggatttttatgatatagtatgcttatgtattttgtactgaaagcatatcctgcttcattgggatattactgaaagcatttaactacatgtaaactcacttgatgatcaataaacttgattttgcaggtggcttcagaattggcacgtggacgaagaaactagggtcaacagaaataacgcacttaaagtaatccatccatccgaggatattttaacagccctgatgaccatcgatgcagagttgactatccctccgtatgagaatcaaaacaacaggcgtcctccaaaagatcaaaccttgtggctcaaccctcagtctttgaatgagcaatatgggagccaatggcgagtgtgggtcaataaactccgtaagaggaatccggagttagcagaaggaatcgctccggtcctcgaatttacggatagaagatcaaggcttaagacaaacaagcagaggtaagttgttacttatgattgttttcctctctgctacatgtattttgttgttcatttctgtaagatataagaattgagttttcctctgatgatattattaggttaaccgatacttctttgtacgccgatagttacttcctgcaaagactcttggacagatctcgaatacatgacacctatgccttgcgagcaattagcaaaaacttcaaaagcgagaagttggagaagttccgttggaacttgaagcaggaccttggggatcagcacaccgagaaatttctcgattttacccagaagtactaccaagaagttgagagggctaaaagtggaatttgggaacaagaatccgcatcattgcttgagaaggctgatatcaatccaccgtctaagcgtaagattttaaacagacttgtcgggaacatcttgggtgtggagatgtctgctgaggagcttacaacttttcttagtgatgtttggacaaaaaaagtacatggcccgtctactgtgaaaagtatatgtaaagcagcagaggacttgaggaagcaaaatggaaatttgtttaatatgtatattcagagcgtccgatatagggcctccgtagaagctggggccgaaaagaagttcaaaggcctcgataaagaaatttggcaattgcttgtgaaagttgagaaggcagccgacgtcatatcaggtaacattccttagttacctttcttttctttttccatcataagtttatagattgtacatgctttgagatttttctttgcaaacaatctcaggtagcatttcagctactgaaacacaaaaacaacgtttttccaacacgttcagtttagctcagctttacacattgatagaaacggataggaacggattctcaaaagtctctgcagctgcccatatggaattggcttggcgtatgacaatgataccagttgacgacaaagaagccgctaggtgcagtagacttcctgcagacagctctcgaccgtttgatggggtcctcagacgtcttttggaaagacaagcatatgaaattgccaccctcaaatcaggacagataaaagagagcggtgtcagagactctgaaataagtattccagttgtagtagaggagaacagattcactttctccattggacttgctgatgtgaagaaagatgggtccaaaagaaagaagcttttatctctgggagagaagcagttagagaaatggcaggagaaaaatgagcgaattagacaagggggctccggtttatgcccgtataaaggtacgattttggacaaggacgctgaactggatcatatcatcccgaggtgctcttgaaattggaactcttcttttgttgtctaaacctatcaatttctttgcggaaatttatttgaagctgtagagttaaaattgagtcttttaaacttttgtaggtcctatagtcgtgacgcctccggaactatttttaatagcgaggctaatttaatatacgccagcaggcgaggaaaccaggagaagaaggaccaaagatacggcatatcagatctcgcccctaattacttgaaggcagtttatggaacctccgactccgccgagatcacaaggattattgaggcttcagtggcttctataaaaaaggatttccttttctctgaactcgagggtgaccagcaacgtgatgtcagacatgcattgttccttgagagagattccaaagccttcgagaaggtgttccgtcgattggccacccaacagtcagctcgtgttaacggtacgcaagcctggcttgcccgtaaactcattagtgtactgaagtcacaactgaagagctggttgtccgagactgggaatacgatagttttcaacttgtgtaaagccgatgctcaacagacttccttcgttcgaaccggactcgctgtgacgaagcctgaaacaacgaagggggagcgtcagggtgtcggctctcatgctatcgatgcttactgtgccttctccgtcgcagcagccgaagggatgcacgaaactttggcacagggtgccggcctcatggaagatactgagtggcttgcaacagcactcccggtcgatgtcgatgtcaactgggtcaagcgtctgccgttgtataggaaaagcgaattatctacaagacctatcttcaaagagggtatctatgccgaatctttcctcaccacctggatctcagagaagggaatagagtcaggcttcagcttgggctctaatagtgtgcagtggcaaggcaaagacacaagagggttattagagttattagcccctttcgccactaaaaatctcaatgtagatacggctttggctagtccgaggcccgtgcaattggacatcagtaaggaaaaagcatttaagcactttgaaatggttgccaaggctccgcatagcgaggtaagaggtcaaaaggtttccgcaatgatccctctttttttgtttctctagtttcaagaatttgggtatatgactaacttctgagtgttccttgatgcatatttgtgatgagacaaatgtttgttctatgttttaggtggatcttcaccaggccgatatattggatgctttgaggtactgcacagccaagaaggatatttccagccgtctgattgatgtccagaagaaaactttaaagaagcccgaagaagtgcttaaggcaaaagatatatacgtcaaggtagacgttgacgtcaaaggcttaggaaagcttaaaggcaaagtaactcaccctgccattgaacaatggaagcgattgtttctcataccagacattgaaacgcgtataggggagaaagccgtcggcattaattggcagcagattggcgagaaatacttcggcgaaggcagcagccgaccacatagcaaaacgaggagagtgtactcacttcctatagtcgattcacccgatgggggttatcgtataaagagaatcgctcctgacgggtctactatttggcaattgacgtctatcaaagatactggttctagtggctttactgtaaatgataagggtgtcaactggaaacagccagtggctatacccgcccttagagacagctcagtagtgggcgtaggtaaagcaactgtgttttaatcaatttcttgtcaggatatatggattataacttaatttttgagaaatctgtagtatttggcgtgaaatgagtttgctttttggtttctcccgtgttataggtgagagataccagccggtcccagaacaacaagtgtactttgatgattggaaatgtgtcgatatcactgatgaacgagtgctctcagtatctgttgcccccgggacgaaggatcgacgatacgtatctgtatcacaaacactgagtgactttaaggcttggctcacagagtccggaataaagctgcattcaccttttgagattccttcccgtgttaaagtggacgctgcaaagtttcagagtgcacatggcatagacgtactcgggaaacctaaaagcaacttgttcataagcaaagtaggcgatgtagtaaattattggtacattagggagtctagtccagtggttataaaccaatattacgacaaggcattactggctgagagagaggcagtcaacgaaacagaaccatgtgatataggcggtgacagtcgtgccgatccaaaaaagaagaggaaggtctaagcttcggccatgctagagtccgcaaaaatcaccagtctctctctacaaatctatctctctctatttttctccagaataatgtgtgagtagttcccagataagggaattagggttcttatagggtttcgctcatgtgttgagcatataagaaacccttagtatgtatttgtatttgtaaaatacttctatcaataaaatttctaattcctaaaaccaaaatccagtgacctcgct

SEQ ID NO: 34 - DNA, 6737 bp, synthetic construct
  source 1..6737: mol_type = other DNA
gtcatgagacgaattctgacaggatatattggcgggtaaacctaagagaaaagagcgtttattagaataatcggatatttaaaagggcgtgaaaaggtttatccgttcgtccatttgtatgtgcatgccaaccacagggttcccctcgggatcaaagtactttgatccaacccctccgctgctatagtgcagtcggcttctgacgttcagtgcagccgtcatctgaaaacgacatgtcgcacaagtcctaagttacgcgacaggctgccgccctgcccttttcctggcgttttcttgtcgcgtgttttagtcgcataaagtagaatacttgcgactagaaccggagacattacgccatgaacaagagcgccgccgctggcctgctgggctatgcccgcgtcagcaccgacgaccaggacttgaccaaccaacgggccgaactgcacgcggccggctgcaccaagctgttttccgagaagatcaccggcaccaggcgcgaccgcccggagctggccaggatgcttgaccacctacgccctggcgacgttgtgacagtgaccaggctagaccgcctggcccgcagcacccgcgacctactggacattgccgagcgcatccaggaggccggcgcgggcctgcgtagcctggcagagccgtgggccgacaccaccacgccggccggccgcatggtgttgaccgtgttcgccggcattgccgagttcgagcgttccctaatcatcgaccgcacccggagcgggcgcgaggccgccaaggcccgaggcgtgaagtttggcccccgccctaccctcaccccggcacagatcgcgcacgcccgcgagctgatcgaccaggaaggccgcaccgtgaaagaggcggctgcactgcttggcgtgcatcgctcgaccctgtaccgcgcacttgagcgcagcgaggaagtgacgcccaccgaggccaggcggcgcggtgccttccgtgaggacgcattgaccgaggccgacgccctggcggccgccgagaatgaacgccaagaggaacaagcatgaaaccgcaccaggacggccaggacgaaccgtttttcattaccgaagagatcgaggcggagatgatcgcggccgggtacgtgttcgagccgcccgcgcacctctcaaccgtgcggctgcatgaaatcctggccggtttgtctgatgccaagctggcggcctggccggccagcttggccgctgaagaaaccgagcgccgccgtctaaaaaggtgatgtgtatttgagtaaaacagcttgcgtcatgcggtcgctgcgtatatgatccgatgagtaaataaacaaatacgcaaggggaacgcatgaaggttatcgctgtacttaaccagaaaggcgggtcaggcaagacgaccatcggaacccatctagcccgcgccctgcaactcgccggggccgatgttctgttagtcgattccgatccccagggcagtgcccgcgattgggcggccgtgcgggaagatcaaccgctaaccgttgtcggcatcgaccgcccgacgattgaccgcgacgtgaaggccatcggccggcgcgacttcgtagtgatcgacggagcgccccaggcggcggacttggctgtgtccgcgatcaaggcagccgacttcgtgctgattccggtgcagccaagcccttacgacatatgggccaccgccgacctggtggagctggttaagcagcgcattgaggtcacggatggaaggctacaagcggcctttgtcgtgtcgcgggcgatcaaaggcacgcgcatcggcggtgaggttgccgaggcgctggccgggtacgagctgcccattcttgagtcccgtatcacgcagcgcgtgagctacccaggcactgccgccgccggcacaaccgttcttgaatcagaacccgagggcgacgctgcccgcgaggtccaggcgctggccgctgaaattaaatcaaaactcatttgagttaatgaggtaaagagaaaatgagcaaaagcacaaacacgctaagtgccggccgtccgagcgcacgcagcagcaaggctgcaacgttggccagcctggcagacacgccagccatgaagcgggtcaactttcagttgccggcggaggatcacaccaagctgaagatgtacgcggtacgccaaggcaagaccattaccgagctgctatctgaatagatcgcgcagctaccagagtaaatgagcaaatgaataaatgagtagatgaattttagcggctaaaggaggcggcatggaaaatcaagaacaaccaggcaccgacgccgtggaatgccccatgtgtggaggaacgggcggttggccaggcgtaagcggctgggttgtctgccggccctgcaatggcactggaacccccaagcccgaggaatcggcgtgacggtcgcaaaccatccggcccggtacaaatcggcgcggcgctgggtgatgacctggtggagaagttgaaggccgcgcaggccgcccagcggcaacgcatcgaggcagaagcacgccccggtgaatcgtggcaagcggccgctgatcgaatccgcaaagaatcccggcaaccgccggcagccggtgcgccgtcgattaggaagccgcccaagggcgacgagcaaccagattttttcgttccgatgctctatgacgtgggcacccgcgatagtcgcagcatcatggacgtggccgttttccgtctgtcgaagcgtgaccgacgagctggcgaggtgatccgctacgagcttccagacgggcacgtagaggtttccgcagggccggccggcatggccagtgtgtgggattacgacctggtactgatggcggtttcccatctaaccgaatccatgaaccgataccgggaagggaagggagacaagcccggccgcgtgttccgtccacacgttgcggacgtactcaagttctgccggcgagccgatggcggaaagcagaaagacgacctggtagaaacctgcattcggttaaacaccacgcacgttgccatgcagcgtacgaagaaggccaagaacggccgcctggtgacggtatccgagggtgaagccttgattagccgctacaagatcgtaaagagcgaaaccgggcggccggagtacatcgagatcgagctagctgattggatgtaccgcgagatcacagaaggcaagaacccggacgtgctgacggttcaccccgattactttttgatcgatcccggcatcggccgttttctctaccgcctggcacgccgcgccgcaggcaaggcagaagccagatggttgttcaagacgatctacgaacgcagtggcagcgccggagagttcaagaagttctgtttcaccgtgcgcaagctgatcgggtcaaatgacctgccggagtacgatttgaaggaggaggcggggcaggctggcccgatcctagtcatgcgctaccgcaacctgatcgagggcgaagcatccgccggttcctaatgtacggagcagatgctagggcaaattgccctagcaggggaaaaaggtcgaaaaggactctttcctgtggatagcacgtacattgggaacccaaagccgtacattgggaaccggaacccgtacattgggaacccaaagccgtacattgggaaccggtcacacatgtaagtgactgatataaaagagaaaaaaggcgatttttccgcctaaaactctttaaaacttattaaaactcttaaaacccgcctggcctgtgcataactgtctggccagcgcacagccgaagagctgcaaaaagcgcctacccttcggtcgctgcgctccctacgccccgccgcttcgcgtcggcctatcgcggccgctggccgctcaaaaatggctggcctacggccaggcaatctaccagggcgcggacaagccgcgccgtcgccactcgaccgccggcgcccacatcaaggcaccctgcctcgcgcgtttcggtgatgacggtgaaaacctctgacacatgcagctcccggtgacggtcacagcttgtctgtaagcggatgccgggagcagacaagcccgtcagggcgcgtcagcgggtgttggcgggtgtcggggcgcagccatgacccagtcacgtagcgatagcggagtgtatactggcttaactatgcggcatcagagcagattgtactgagagtgcaccatatgcggtgtgaaataccgcacagatgcgtaaggagaaaataccgcatcaggcgctcttccgcttcctcgctcactgactcgctgcgctcggtcgttcggctgcggcgagcggtatcagctcactcaaaggcggtaatacggttatccacagaatcaggggataacgcaggaaagaacatgtgagcaaaaggccagcaaaaggccaggaaccgtaaaaaggccgcgttgctggcgtttttccataggctccgcccccctgacgagcatcacaaaaatcgacgctcaagtcagaggtggcgaaacccgacaggactataaagataccaggcgtttccccctggaagctccctcgtgcgctctcctgttccgaccctgccgcttaccggatacctgtccgcctttctcccttcgggaagcgtggcgctttctcatagctcacgctgtaggtatctcagttcggtgtaggtcgttcgctccaagctgggctgtgtgcacgaaccccccgttcagcccgaccgctgcgccttatccggtaactatcgtcttgagtccaacccggtaagacacgacttatcgccactggcagcagccactggtaacaggattagcagagcgaggtatgtaggcggtgctacagagttcttgaagtggtggcctaactacggctacactagaaggacagtatttggtatctgcgctctgctgaagccagttaccttcggaaaaagagttggtagctcttgatccggcaaacaaaccaccgctggtagcggtggtttttttgtttgcaagcagcagattacgcgcagaaaaaaaggatctcaagaagatcctttgatcttttctacggggtctgacgctcagtggaacgaaaactcacgttaagggattttggtcatgcattctaggtgattagaaaaactcatcgagcatcaaatgaaactgcaatttattcatatcaggattatcaataccatatttttgaaaaagccgtttctgtaatgaaggagaaaactcaccgaggcagttccataggatggcaagatcctggtatcggtctgcgattccgactcgtccaacatcaatacaacctattaatttcccctcgtcaaaaataaggttatcaagtgagaaatcaccatgagtgacgactgaatccggtgagaatggcaaaagtttatgcatttctttccagacttgttcaacaggccagccattacgctcgtcatcaaaatcactcgcatcaaccaaaccgttattcattcgtgattgcgcctgagcgagtcgaaatacgcgatcgctgttaaaaggacaattacaaacaggaatcgaatgcaaccggcgcaggaacactgccagcgcatcaacaatattttcacctgaatcaggatattcttctaatacctggaatgctgttttccctgggatcgcagtggtgagtaaccatgcatcatcaggagtacggataaaatgcttgatggtcggaagaggcataaattccgtcagccagtttagtctgaccatctcatctgtaacatcattggcaacgctacctttgccatgtttcagaaacaactctggcgcatcgggcttcccatacaatcggtagattgtcgcacctgattgcccgacattatcgcgagcccatttatacccatataaatcagcatccatgttggaatttaatcgcggccttgagcaagacgtttcccgttgaatatggctcataacagaacttattatttccttcctcttttctacagtatttaaagataccccaagaagctaattataacaagacgaactccaattcactgttccttgcattctaaaaccttaaataccagaaaacagctttttcaaagttgttttcaaagttggcgtataacatagtatcgacggagccgattttgaaaccgcggtgatcacaggcagcaacgctctgtcatcgttacaatcaacatgctaccctccgcgagatcatccgtgtttcaaacccggcagcttagttgccgttcttccgaatagcatcggtaacatgagcaaagtctgccgccttacaacggctctcccgctgacgccgtcccggactgatgggctgcctgtatcgagtggtgattttgtgccgagctgccggtcggggagctgttggctggctggtggcaggatatattgtggtgtaaacataacgaattcgtctcaggagcatcttcattcttaagatatgaagataatcttcaaaaggcccctgggaatctgaaagaagagaagcaggcccatttatatgggaaagaacaatagtatttcttatataggcccatttaagttgaaaacaatcttcaaaagtcccacatcgcttagataagaaaacgaagctgagtttatatacagctagagtcgaagtagtgattgttggtagtagcgactccatggtttcagttgcaggtttattgggatagggaaacctatcccaataggcctgattgaagtcgcccacgggcgagctgaaatcatctaaaatcatgactgactccggcacctgcttcggcatccggggtttttctttttcgct

SEQ ID NO: 35 - DNA, 6737 bp, synthetic construct
  source 1..6737: mol_type = other DNA
gtcatgagacgaattctgacaggatatattggcgggtaaacctaagagaaaagagcgtttattagaataatcggatatttaaaagggcgtgaaaaggtttatccgttcgtccatttgtatgtgcatgccaaccacagggttcccctcgggatcaaagtactttgatccaacccctccgctgctatagtgcagtcggcttctgacgttcagtgcagccgtcatctgaaaacgacatgtcgcacaagtcctaagttacgcgacaggctgccgccctgcccttttcctggcgttttcttgtcgcgtgttttagtcgcataaagtagaatacttgcgactagaaccggagacattacgccatgaacaagagcgccgccgctggcctgctgggctatgcccgcgtcagcaccgacgaccaggacttgaccaaccaacgggccgaactgcacgcggccggctgcaccaagctgttttccgagaagatcaccggcaccaggcgcgaccgcccggagctggccaggatgcttgaccacctacgccctggcgacgttgtgacagtgaccaggctagaccgcctggcccgcagcacccgcgacctactggacattgccgagcgcatccaggaggccggcgcgggcctgcgtagcctggcagagccgtgggccgacaccaccacgccggccggccgcatggtgttgaccgtgttcgccggcattgccgagttcgagcgttccctaatcatcgaccgcacccggagcgggcgcgaggccgccaaggcccgaggcgtgaagtttggcccccgccctaccctcaccccggcacagatcgcgcacgcccgcgagctgatcgaccaggaaggccgcaccgtgaaagaggcggctgcactgcttggcgtgcatcgctcgaccctgtaccgcgcacttgagcgcagcgaggaagtgacgcccaccgaggccaggcggcgcggtgccttccgtgaggacgcattgaccgaggccgacgccctggcggccgccgagaatgaacgccaagaggaacaagcatgaaaccgcaccaggacggccaggacgaaccgtttttcattaccgaagagatcgaggcggagatgatcgcggccgggtacgtgttcgagccgcccgcgcacctctcaaccgtgcggctgcatgaaatcctggccggtttgtctgatgccaagctggcggcctggccggccagcttggccgctgaagaaaccgagcgccgccgtctaaaaaggtgatgtgtatttgagtaaaacagcttgcgtcatgcggtcgctgcgtatatgatccgatgagtaaataaacaaatacgcaaggggaacgcatgaaggttatcgctgtacttaaccagaaaggcgggtcaggcaagacgaccatcggaacccatctagcccgcgccctgcaactcgccggggccgatgttctgttagtcgattccgatccccagggcagtgcccgcgattgggcggccgtgcgggaagatcaaccgctaaccgttgtcggcatcgaccgcccgacgattgaccgcgacgtgaaggccatcggccggcgcgacttcgtagtgatcgacggagcgccccaggcggcggacttggctgtgtccgcgatcaaggcagccgacttcgtgctgattccggtgcagccaagcccttacgacatatgggccaccgccgacctggtggagctggttaagcagcgcattgaggtcacggatggaaggctacaagcggcctttgtcgtgtcgcgggcgatcaaaggcacgcgcatcggcggtgaggttgccgaggcgctggccgggtacgagctgcccattcttgagtcccgtatcacgcagcgcgtgagctacccaggcactgccgccgccggcacaaccgttcttgaatcagaacccgagggcgacgctgcccgcgaggtccaggcgctggccgctgaaattaaatcaaaactcatttgagttaatgaggtaaagagaaaatgagcaaaagcacaaacacgctaagtgccggccgtccgagcgcacgcagcagcaaggctgcaacgttggccagcctggcagacacgccagccatgaagcgggtcaactttcagttgccggcggaggatcacaccaagctgaagatgtacgcggtacgccaaggcaagaccattaccgagctgctatctgaatagatcgcgcagctaccagagtaaatgagcaaatgaataaatgagtagatgaattttagcggctaaaggaggcggcatggaaaatcaagaacaaccaggcaccgacgccgtggaatgccccatgtgtggaggaacgggcggttggccaggcgtaagcggctgggttgtctgccggccctgcaatggcactggaacccccaagcccgaggaatcggcgtgacggtcgcaaaccatccggcccggtacaaatcggcgcggcgctgggtgatgacctggtggagaagttgaaggccgcgcaggccgcccagcggcaacgcatcgaggcagaagcacgccccggtgaatcgtggcaagcggccgctgatcgaatccgcaaagaatcccggcaaccgccggcagccggtgcgccgtcgattaggaagccgcccaagggcgacgagcaaccagattttttcgttccgatgctctatgacgtgggcacccgcgatagtcgcagcatcatggacgtggccgttttccgtctgtcgaagcgtgaccgacgagctggcgaggtgatccgctacgagcttccagacgggcacgtagaggtttccgcagggccggccggcatggccagtgtgtgggattacgacctggtactgatggcggtttcccatctaaccgaatccatgaaccgataccgggaagggaagggagacaagcccggccgcgtgttccgtccacacgttgcggacgtactcaagttctgccggcgagccgatggcggaaagcagaaagacgacctggtagaaacctgcattcggttaaacaccacgcacgttgccatgcagcgtacgaagaaggccaagaacggccgcctggtgacggtatccgagggtgaagccttgattagccgctacaagatcgtaaagagcgaaaccgggcggccggagtacatcgagatcgagctagctgattggatgtaccgcgagatcacagaaggcaagaacccggacgtgctgacggttcaccccgattactttttgatcgatcccggcatcggccgttttctctaccgcctggcacgccgcgccgcaggcaaggcagaagccagatggttgttcaagacgatctacgaacgcagtggcagcgccggagagttcaagaagttctgtttcaccgtgcgcaagctgatcgggtcaaatgacctgccggagtacgatttgaaggaggaggcggggcaggctggcccgatcctagtcatgcgctaccgcaacctgatcgagggcgaagcatccgccggttcctaatgtacggagcagatgctagggcaaattgccctagcaggggaaaaaggtcgaaaaggactctttcctgtggatagcacgtacattgggaacccaaagccgtacattgggaaccggaacccgtacattgggaacccaaagccgtacattgggaaccggtcacacatgtaagtgactgatataaaagagaaaaaaggcgatttttccgcctaaaactctttaaaacttattaaaactcttaaaacccgcctggcctgtgcataactgtctggccagcgcacagccgaagagctgcaaaaagcgcctacccttcggtcgctgcgctccctacgccccgccgcttcgcgtcggcctatcgcggccgctggccgctcaaaaatggctggcctacggccaggcaatctaccagggcgcggacaagccgcgccgtcgccactcgaccgccggcgcccacatcaaggcaccctgcctcgcgcgtttcggtgatgacggtgaaaacctctgacacatgcagctcccggtgacggtcacagcttgtctgtaagcggatgccgggagcagacaagcccgtcagggcgcgtcagcgggtgttggcgggtgtcggggcgcagccatgacccagtcacgtagcgatagcggagtgtatactggcttaactatgcggcatcagagcagattgtactgagagtgcaccatatgcggtgtgaaataccgcacagatgcgtaaggagaaaataccgcatcaggcgctcttccgcttcctcgctcactgactcgctgcgctcggtcgttcggctgcggcgagcggtatcagctcactcaaaggcggtaatacggttatccacagaatcaggggataacgcaggaaagaacatgtgagcaaaaggccagcaaaaggccaggaaccgtaaaaaggccgcgttgctggcgtttttccataggctccgcccccctgacgagcatcacaaaaatcgacgctcaagtcagaggtggcgaaacccgacaggactataaagataccaggcgtttccccctggaagctccctcgtgcgctctcctgttccgaccctgccgcttaccggatacctgtccgcctttctcccttcgggaagcgtggcgctttctcatagctcacgctgtaggtatctcagttcggtgtaggtcgttcgctccaagctgggctgtgtgcacgaaccccccgttcagcccgaccgctgcgccttatccggtaactatcgtcttgagtccaacccggtaagacacgacttatcgccactggcagcagccactggtaacaggattagcagagcgaggtatgtaggcggtgctacagagttcttgaagtggtggcctaactacggctacactagaaggacagtatttggtatctgcgctctgctgaagccagttaccttcggaaaaagagttggtagctcttgatccggcaaacaaaccaccgctggtagcggtggtttttttgtttgcaagcagcagattacgcgcagaaaaaaaggatctcaagaagatcctttgatcttttctacggggtctgacgctcagtggaacgaaaactcacgttaagggattttggtcatgcattctaggtgattagaaaaactcatcgagcatcaaatgaaactgcaatttattcatatcaggattatcaataccatatttttgaaaaagccgtttctgtaatgaaggagaaaactcaccgaggcagttccataggatggcaagatcctggtatcggtctgcgattccgactcgtccaacatcaatacaacctattaatttcccctcgtcaaaaataaggttatcaagtgagaaatcaccatgagtgacgactgaatccggtgagaatggcaaaagtttatgcatttctttccagacttgttcaacaggccagccattacgctcgtcatcaaaatcactcgcatcaaccaaaccgttattcattcgtgattgcgcctgagcgagtcgaaatacgcgatcgctgttaaaaggacaattacaaacaggaatcgaatgcaaccggcgcaggaacactgccagcgcatcaacaatattttcacctgaatcaggatattcttctaatacctggaatgctgttttccctgggatcgcagtggtgagtaaccatgcatcatcaggagtacggataaaatgcttgatggtcggaagaggcataaattccgtcagccagtttagtctgaccatctcatctgtaacatcattggcaacgctacctttgccatgtttcagaaacaactctggcgcatcgggcttcccatacaatcggtagattgtcgcacctgattgcccgacattatcgcgagcccatttatacccatataaatcagcatccatgttggaatttaatcgcggccttgagcaagacgtttcccgttgaatatggctcataacagaacttattatttccttcctcttttctacagtatttaaagataccccaagaagctaattataacaagacgaactccaattcactgttccttgcattctaaaaccttaaataccagaaaacagctttttcaaagttgttttcaaagttggcgtataacatagtatcgacggagccgattttgaaaccgcggtgatcacaggcagcaacgctctgtcatcgttacaatcaacatgctaccctccgcgagatcatccgtgtttcaaacccggcagcttagttgccgttcttccgaatagcatcggtaacatgagcaaagtctgccgccttacaacggctctcccgctgacgccgtcccggactgatgggctgcctgtatcgagtggtgattttgtgccgagctgccggtcggggagctgttggctggctggtggcaggatatattgtggtgtaaacataacgaattcgtctcaggagcatcttcattcttaagatatgaagataatcttcaaaaggcccctgggaatctgaaagaagagaagcaggcccatttatatgggaaagaacaatagtatttcttatataggcccatttaagttgaaaacaatcttcaaaagtcccacatcgcttagataagaaaacgaagctgagtttatatacagctagagtcgaagtagtgattgcttcttgctaaagctaacaggtttcagttgcaggtttattgggatagggaaacctatcccaataggcctgattgaagtcgcccacgggcgagctgaaatcatctaaaatcatgactgactccggcacctgcttcggcatccggggtttttctttttcgct

SEQ ID NO: 36 - DNA, 8420 bp, synthetic construct
  source 1..8420: mol_type = other DNA
ggagactagagccaagctgatctcctttgccccggagatcaccatggacgactttctctatctctacgatctaggaagaaagttcgacggagaaggtgacgataccatgttcaccaccgataatgagaagattagcctcttcaatttcagaaagaatgctgacccacagatggttagagaggcctacgcggcaggtctgatcaagacgatctacccgagtaataatctccaggagatcaaataccttcccaagaaggttaaagatgcagtcaaaagattcaggactaactgcatcaagaacacagagaaagatatatttctcaagatcagaagtactattccagtatggacgattcaaggcttgcttcataaaccaaggcaagtaatagagattggagtctctaagaaagtagttcctactgaatcaaaggccatggagtcaaaaattcagatcgaggatctaacagaactcgccgtgaagactggcgaacagttcatacagagtcttttacgactcaatgacaagaagaaaatcttcgtcaacatggtggagcacgacactctcgtctactccaagaatatcaaagatacagtctcagaagaccaaagggctattgagacttttcaacaaagggtaatatcgggaaacctcctcggattccattgcccagctatctgtcacttcatcaaaaggacagtagaaaaggaaggtggcacctacaaatgccatcattgcgataaaggaaaggctatcgttcaagatgcctctgccgacagtggtcccaaagatggacccccacccacgaggagcatcgtggaaaaagaagacgttccaaccacgtcttcaaagcaagtggattgatgtgatatctccactgacgtaagggatgacgcacaatcccactatccttcgcaagacccttcctctatataaggaagttcatttcatttggagaggactccggtatttttacaacaataccacaacaaaacaaacaacaaacaacattacaatttactattctagtcgaaatggaacgagctatacaaggaaacgacgctagggaacaagctaacagtgaacgttgggatggaggatcaggaggtaccacttctcccttcaaacttcctgacgaaagtccgagttggactgagtggcggctacataacgatgagactaattcgaatcaagataatccccttggtttcaaggaaagctggggtttcgggaaagttgtatttaagagatatctcagatacgacaggacggaagcttcactgcacagagtccttggatcttggacgggagattcggttaactatgcagcatctcgatttttcggtttcgaccagatcggatgtacctatagtattcggtttcgaggagttagtatcaccgtttctggaggctctcgaactcttcagcatctctgtgagatggcaattcggtctaagcaagaactgctacagcttgccccaatcgaagtggaaagtaatgtatcaagaggatgccctgaaggtactgaaaccttcgaaaaagaaagcgagtgagcttggaatggatcttcgatcccgatcgttcaaacatttggcaataaagtttcttaagattgaatcctgttgccggtcttgcgacgattatcatataatttctgttgaattacgttaagcatgtaataattaacatgtaatgcatgacgttatttatgagatgggtttttatgattagagtcccgcaattatacatttaatacgcgatagaaaacaaaatatagcgcgcaaactaggataaattatcgcgcdcggtgtcatctatgttactagatcgggaattgccaagctaattcttgaagacgaaagggcctcgtgatacgcctatttttataggttaatgtcatgataataatggtttcttagacgtcaggtggcacttttcggggaaatgtgcgcggaacccctatttgtttatttttctaaatacattcaaatatgtatccgctcatgagacaataaccctgataaatgcttcaataatgggaccgactcgcgcttgagacgaagctttgacaggatatattggcgggtaaacctaagagaaaagagcgtttattagaataatcggatatttaaaagggcgtgaaaaggtttatccgttcgtccatttgtatgtgcatgccaaccacagggttcccctcgggatcaaagtactttgatccaacccctccgctgctatagtgcagtcggcttctgacgttcagtgcagccgtcatctgaaaacgacatgtcgcacaagtcctaagttacgcgacaggctgccgccctgcccttttcctggcgttttcttgtcgcgtgttttagtcgcataaagtagaatacttgcgactagaaccggagacattacgccatgaacaagagcgccgccgctggcctgctgggctatgcccgcgtcagcaccgacgaccaggacttgaccaaccaacgggccgaactgcacgcggccggctgcaccaagctgttttccgagaagatcaccggcaccaggcgcgaccgcccggagctggccaggatgcttgaccacctacgccctggcgacgttgtgacagtgaccaggctagaccgcctggcccgcagcacccgcgacctactggacattgccgagcgcatccaggaggccggcgcgggcctgcgtagcctggcagagccgtgggccgacaccaccacgccggccggccgcatggtgttgaccgtgttcgccggcattgccgagttcgagcgttccctaatcatcgaccgcacccggagcgggcgcgaggccgccaaggcccgaggcgtgaagtttggcccccgccctaccctcaccccggcacagatcgcgcacgcccgcgagctgatcgaccaggaaggccgcaccgtgaaagaggcggctgcactgcttggcgtgcatcgctcgaccctgtaccgcgcacttgagcgcagcgaggaagtgacgcccaccgaggccaggcggcgcggtgccttccgtgaggacgcattgaccgaggccgacgccctggcggccgccgagaatgaacgccaagaggaacaagcatgaaaccgcaccaggacggccaggacgaaccgtttttcattaccgaagagatcgaggcggagatgatcgcggccgggtacgtgttcgagccgcccgcgcacctctcaaccgtgcggctgcatgaaatcctggccggtttgtctgatgccaagctggcggcctggccggccagcttggccgctgaagaaaccgagcgccgccgtctaaaaaggtgatgtgtatttgagtaaaacagcttgcgtcatgcggtcgctgcgtatatgatccgatgagtaaataaacaaatacgcaaggggaacgcatgaaggttatcgctgtacttaaccagaaaggcgggtcaggcaagacgaccatcggaacccatctagcccgcgccctgcaactcgccggggccgatgttctgttagtcgattccgatccccagggcagtgcccgcgattgggcggccgtgcgggaagatcaaccgctaaccgttgtcggcatcgaccgcccgacgattgaccgcgacgtgaaggccatcggccggcgcgacttcgtagtgatcgacggagcgccccaggcggcggacttggctgtgtccgcgatcaaggcagccgacttcgtgctgattccggtgcagccaagcccttacgacatatgggccaccgccgacctggtggagctggttaagcagcgcattgaggtcacggatggaaggctacaagcggcctttgtcgtgtcgcgggcgatcaaaggcacgcgcatcggcggtgaggttgccgaggcgctggccgggtacgagctgcccattcttgagtcccgtatcacgcagcgcgtgagctacccaggcactgccgccgccggcacaaccgttcttgaatcagaacccgagggcgacgctgcccgcgaggtccaggcgctggccgctgaaattaaatcaaaactcatttgagttaatgaggtaaagagaaaatgagcaaaagcacaaacacgctaagtgccggccgtccgagcgcacgcagcagcaaggctgcaacgttggccagcctggcagacacgccagccatgaagcgggtcaactttcagttgccggcggaggatcacaccaagctgaagatgtacgcggtacgccaaggcaagaccattaccgagctgctatctgaatagatcgcgcagctaccagagtaaatgagcaaatgaataaatgagtagatgaattttagcggctaaaggaggcggcatggaaaatcaagaacaaccaggcaccgacgccgtggaatgccccatgtgtggaggaacgggcggttggccaggcgtaagcggctgggttgtctgccggccctgcaatggcactggaacccccaagcccgaggaatcggcgtgacggtcgcaaaccatccggcccggtacaaatcggcgcggcgctgggtgatgacctggtggagaagttgaaggccgcgcaggccgcccagcggcaacgcatcgaggcagaagcacgccccggtgaatcgtggcaagcggccgctgatcgaatccgcaaagaatcccggcaaccgccggcagccggtgcgccgtcgattaggaagccgcccaagggcgacgagcaaccagattttttcgttccgatgctctatgacgtgggcacccgcgatagtcgcagcatcatggacgtggccgttttccgtctgtcgaagcgtgaccgacgagctggcgaggtgatccgctacgagcttccagacgggcacgtagaggtttccgcagggccggccggcatggccagtgtgtgggattacgacctggtactgatggcggtttcccatctaaccgaatccatgaaccgataccgggaagggaagggagacaagcccggccgcgtgttccgtccacacgttgcggacgtactcaagttctgccggcgagccgatggcggaaagcagaaagacgacctggtagaaacctgcattcggttaaacaccacgcacgttgccatgcagcgtacgaagaaggccaagaacggccgcctggtgacggtatccgagggtgaagccttgattagccgctacaagatcgtaaagagcgaaaccgggcggccggagtacatcgagatcgagctagctgattggatgtaccgcgagatcacagaaggcaagaacccggacgtgctgacggttcaccccgattactttttgatcgatcccggcatcggccgttttctctaccgcctggcacgccgcgccgcaggcaaggcagaagccagatggttgttcaagacgatctacgaacgcagtggcagcgccggagagttcaagaagttctgtttcaccgtgcgcaagctgatcgggtcaaatgacctgccggagtacgatttgaaggaggaggcggggcaggctggcccgatcctagtcatgcgctaccgcaacctgatcgagggcgaagcatccgccggttcctaatgtacggagcagatgctagggcaaattgccctagcaggggaaaaaggtcgaaaaggactctttcctgtggatagcacgtacattgggaacccaaagccgtacattgggaaccggaacccgtacattgggaacccaaagccgtacattgggaaccggtcacacatgtaagtgactgatataaaagagaaaaaaggcgatttttccgcctaaaactctttaaaacttattaaaactcttaaaacccgcctggcctgtgcataactgtctggccagcgcacagccgaagagctgcaaaaagcgcctacccttcggtcgctgcgctccctacgccccgccgcttcgcgtcggcctatcgcggccgctggccgctcaaaaatggctggcctacggccaggcaatctaccagggcgcggacaagccgcgccgtcgccactcgaccgccggcgcccacatcaaggcaccctgcctcgcgcgtttcggtgatgacggtgaaaacctctgacacatgcagctcccggtgacggtcacagcttgtctgtaagcggatgccgggagcagacaagcccgtcagggcgcgtcagcgggtgttggcgggtgtcggggcgcagccatgacccagtcacgtagcgatagcggagtgtatactggcttaactatgcggcatcagagcagattgtactgagagtgcaccatatgcggtgtgaaataccgcacagatgcgtaaggagaaaataccgcatcaggcgctcttccgcttcctcgctcactgactcgctgcgctcggtcgttcggctgcggcgagcggtatcagctcactcaaaggcggtaatacggttatccacagaatcaggggataacgcaggaaagaacatgtgagcaaaaggccagcaaaaggccaggaaccgtaaaaaggccgcgttgctggcgtttttccataggctccgcccccctgacgagcatcacaaaaatcgacgctcaagtcagaggtggcgaaacccgacaggactataaagataccaggcgtttccccctggaagctccctcgtgcgctctcctgttccgaccctgccgcttaccggatacctgtccgcctttctcccttcgggaagcgtggcgctttctcatagctcacgctgtaggtatctcagttcggtgtaggtcgttcgctccaagctgggctgtgtgcacgaaccccccgttcagcccgaccgctgcgccttatccggtaactatcgtcttgagtccaacccggtaagacacgacttatcgccactggcagcagccactggtaacaggattagcagagcgaggtatgtaggcggtgctacagagttcttgaagtggtggcctaactacggctacactagaaggacagtatttggtatctgcgctctgctgaagccagttaccttcggaaaaagagttggtagctcttgatccggcaaacaaaccaccgctggtagcggtggtttttttgtttgcaagcagcagattacgcgcagaaaaaaaggatctcaagaagatcctttgatcttttctacggggtctgacgctcagtggaacgaaaactcacgttaagggattttggtcatgcattctaggtgattagaaaaactcatcgagcatcaaatgaaactgcaatttattcatatcaggattatcaataccatatttttgaaaaagccgtttctgtaatgaaggagaaaactcaccgaggcagttccataggatggcaagatcctggtatcggtctgcgattccgactcgtccaacatcaatacaacctattaatttcccctcgtcaaaaataaggttatcaagtgagaaatcaccatgagtgacgactgaatccggtgagaatggcaaaagtttatgcatttctttccagacttgttcaacaggccagccattacgctcgtcatcaaaatcactcgcatcaaccaaaccgttattcattcgtgattgcgcctgagcgagtcgaaatacgcgatcgctgttaaaaggacaattacaaacaggaatcgaatgcaaccggcgcaggaacactgccagcgcatcaacaatattttcacctgaatcaggatattcttctaatacctggaatgctgttttccctgggatcgcagtggtgagtaaccatgcatcatcaggagtacggataaaatgcttgatggtcggaagaggcataaattccgtcagccagtttagtctgaccatctcatctgtaacatcattggcaacgctacctttgccatgtttcagaaacaactctggcgcatcgggcttcccatacaatcggtagattgtcgcacctgattgcccgacattatcgcgagcccatttatacccatataaatcagcatccatgttggaatttaatcgcggccttgagcaagacgtttcccgttgaatatggctcataacagaacttattatttccttcctcttttctacagtatttaaagataccccaagaagctaattataacaagacgaactccaattcactgttccttgcattctaaaaccttaaataccagaaaacagctttttcaaagttgttttcaaagttggcgtataacatagtatcgacggagccgattttgaaaccgcggtgatcacaggcagcaacgctctgtcatcgttacaatcaacatgctaccctccgcgagatcatccgtgtttcaaacccggcagcttagttgccgttcttccgaatagcatcggtaacatgagcaaagtctgccgccttacaacggctctcccgctgacgccgtcccggactgatgggctgcctgtatcgagtggtgattttgtgccgagctgccggtcggggagctgttggctggctggtggcaggatatattgtggtgtaaacataacaagcttcgtctcagtca

SEQ ID NO: 37 - DNA, 20 bp, synthetic construct
  source 1..20: mol_type = other DNA
ttggtagtagcgactccatg

SEQ ID NO: 38 - DNA, 20 bp, synthetic construct
  source 1..20: mol_type = other DNA
cttcttgctaaagctaacag

SEQ ID NO: 39 - DNA, 27 bp, Nicotiana sp.
  source 1..27: mol_type = genomic DNA
ggcttaatttactgctatcttgttcaa

SEQ ID NO: 40 - DNA, 26 bp, Nicotiana sp.
  source 1..26: mol_type = genomic DNA
cagttaatcagaaaagaatgtacagg

SEQ ID NO: 41 - DNA, 27 bp, Nicotiana sp.
  source 1..27: mol_type = genomic DNA
ggcttaatttactgctattttgttcag

SEQ ID NO: 42 - DNA, 27 bp, Nicotiana sp.
  source 1..27: mol_type = genomic DNA
ccaaaacagttaataagaaaagaatgc

SEQ ID NO: 43 - DNA, 20 bp, Nicotiana sp.
  source 1..20: mol_type = genomic DNA
ttacgacacgaagtatatag

SEQ ID NO: 44 - DNA, 20 bp, Nicotiana sp.
  source 1..20: mol_type = genomic DNA
aactcgaagatcatgagcag

SEQ ID NO: 45 - DNA, 20 bp, Nicotiana sp.
  source 1..20: mol_type = genomic DNA
ttacgataggaagtatattt

SEQ ID NO: 46 - DNA, 20 bp, Nicotiana sp.
  source 1..20: mol_type = genomic DNA
aactcgaagatcatgatcta

SEQ ID NO: 47 - DNA, 78 bp, Caenorhabditis elegans
  source 1..78: mol_type = genomic DNA
caatacggcaagatgagaatgactggaaaccgtaccgctcgtggtgcctatggtagcggagcttcacatggcttcaga

SEQ ID NO: 48 - DNA, 65 bp, Caenorhabditis elegans
  source 1..65: mol_type = genomic DNA
caatacggcaagatgagaatgactggaaaccgtaccgctcgagcggagcttcacatggcttcaga

SEQ ID NO: 49 - DNA, 71 bp, Caenorhabditis elegans
  source 1..71: mol_type = genomic DNA
caatacggcaagatgagaatgactggaaaccgtaccgctcctatggtagcggagcttcacatggcttcaga

SEQ ID NO: 50 - DNA, 66 bp, Caenorhabditis elegans
  source 1..66: mol_type = genomic DNA
caatacggcaagatgagaatgactggaaaccgtaccgctggtagcggagcttcacatggcttcaga

SEQ ID NO: 51 - DNA, 63 bp, Caenorhabditis elegans
  source 1..63: mol_type = genomic DNA
caatacggcaagatgagaatgactggaaaccgtaccgctagcggagcttcacatggcttcaga

SEQ ID NO: 52 - DNA, 65 bp, Caenorhabditis elegans
  source 1..65: mol_type = genomic DNA
caatacggcaagatgagaatgactggaaaccgtaccgcggtagcggagcttcacatggcttcaga

SEQ ID NO: 53 - DNA, 64 bp, Caenorhabditis elegans
  source 1..64: mol_type = genomic DNA
caatacggcaagatgagaatgactggaaaccgtaccgcgtagcggagcttcacatggcttcaga

SEQ ID NO: 54 - DNA, 59 bp, Caenorhabditis elegans
  source 1..59: mol_type = genomic DNA
caatacggcaagatgagaatgactggaaaccgtaccgcggagcttcacatggcttcaga

SEQ ID NO: 55 - DNA, 70 bp, Caenorhabditis elegans
  source 1..70: mol_type = genomic DNA
caatacggcaagatgagaatgactggaaaccgtacctgcctatggtagcggagcttcacatggcttcaga

SEQ ID NO: 56 - DNA, 59 bp, Caenorhabditis elegans
  source 1..59: mol_type = genomic DNA
caatacggcaagatgagaatgactggaaaccgtacagcggagcttcacatggcttcaga

SEQ ID NO: 57 - DNA, 73 bp, Caenorhabditis elegans
  source 1..73: mol_type = other DNA
caatacggcaagatgagaatgactggaaaccgtaccgactggaaaccgtagcggagcttcacatggcttcaga

SEQ ID NO: 58 - DNA, 89 bp, Caenorhabditis elegans
  source 1..89: mol_type = genomic DNA
caatacggcaagatgagaatgactggaaaccgtaccgctcgtggcggtacggtttccagtctggtagcggagcttcacatggcttcaga

SEQ ID NO: 59 - DNA, 101 bp, Caenorhabditis elegans
  source 1..101: mol_type = genomic DNA
caatacggcaagatgagaatgactggaaaccgtaccgctcggtagcggagcttcacatggcttcagaccaacatggtagcggagcttcacatggcttcaga

SEQ ID NO: 60 - DNA, 48 bp, synthetic construct
  source 1..48: mol_type = other DNA
aaaaggccggcggccacgaaaaaggccggccaggcaaaaaagaaaaag